European Patent Application EP 4 241 786 A2, published September 13, 2023. Title: METHODS AND COMPOSITIONS FOR STIMULATING IMMUNE RESPONSE. Applicant: BioNTech SE. The sequence listing filed with the application follows.

SEQUENCE LISTING (12 sequences)

SEQ ID NO: 1 - RNA, 17 nt, synthetic construct
  misc_feature 1..17: note = Sequence of immunostimulatory RNA molecule
  source 1..17: mol_type = other RNA
aacttctggaggggtga

SEQ ID NO: 2 - RNA, 21 nt, synthetic construct
  misc_feature 1..21: note = Sequence of immunostimulatory RNA molecule
  source 1..21: mol_type = other RNA
aacttctggaggggtgagaat

SEQ ID NO: 3 - skipped

SEQ ID NO: 4 - RNA, 11 nt, synthetic construct
  misc_feature 1..11: note = Sequence of immunostimulatory RNA molecule
  source 1..11: mol_type = other RNA
aagaattgctt

SEQ ID NO: 5 - RNA, 38 nt, synthetic construct
  misc_feature 1..38: note = Sequence of immunostimulatory RNA molecule
  source 1..38: mol_type = other RNA
gggcgaactagtaacttctggaggggtgagaatctcga

SEQ ID NO: 6 - RNA, 23 nt, synthetic construct
  misc_feature 1..23: note = Sequence of immunostimulatory RNA molecule
  source 1..23: mol_type = other RNA
aacttctggaggggtgattgctt

SEQ ID NO: 7 - RNA, 40 nt, synthetic construct
  misc_feature 1..40: note = Sequence of immunostimulatory RNA molecule
  source 1..40: mol_type = other RNA
gggcgaactagtaacttctggaggggtgattgcttctcga

SEQ ID NO: 8 - RNA, 43 nt, synthetic construct
  misc_feature 1..43: note = Sequence of immunostimulatory RNA molecule
  source 1..43: mol_type = other RNA
aacttctggaggggtgagaatggacgaaaaacaagaattgctt

SEQ ID NO: 9 - RNA, 60 nt, synthetic construct
  misc_feature 1..60: note = Sequence of immunostimulatory RNA molecule
  source 1..60: mol_type = other RNA
gggcgaactagtaacttctggaggggtgagaatggacgaaaaacaagaattgcttctcga

SEQ ID NO: 10 - RNA, 32 nt, synthetic construct
  misc_feature 1..32: note = Sequence of immunostimulatory RNA molecule
  source 1..32: mol_type = other RNA
aacttctggaggggtgagaataagaattgctt

SEQ ID NO: 11 - RNA, 49 nt, synthetic construct
  misc_feature 1..49: note = Sequence of immunostimulatory RNA molecule
  source 1..49: mol_type = other RNA
gggcgaactagtaacttctggaggggtgagaataagaattgcttctcga

SEQ ID NO: 12 - RNA, 1565 nt, Influenza A virus
  source 1..1565: mol_type = other RNA
agcaaaagcagggtagataatcactcactgagtgacatcaaaatcatggcgtctcaaggcaccaaacgatcttacgaacagatggagactgatggagaacgccagaatgccactgaaatcagagcatccgtcggaaaaatgattggtggaattggacgattctacatccaaatgtgcaccgaactcaaactcagtgattatgagggacggttgatccaaaacagcttaacaatagagagaatggtgctctctgcttttgacgaaaggagaaataaataccttgaagaacatcccagtgcggggaaagatcctaagaaaactggaggacctatatacaggagagtaaacggaaagtggatgagagaactcatcctttatgacaaagaagaaataaggcgaatctggcgccaagctaataatggtgacgatgcaacggctggtctgactcacatgatgatctggcattccaatttgaatgatgcaacttatcagaggacaagagctcttgttcgcaccggaatggatcccaggatgtgctctctgatgcaaggttcaactctccctaggaggtctggagccgcaggtgctgcagtcaaaggagttggaacaatggtgatggaattggtcagaatgatcaaacgtgggatcaatgatcggaacttctggaggggtgagaatggacgaaaaacaagaattgcttatgaaagaatgtgcaacattctcaaagggaaatttcaaactgctgcacaaaaagcaatgatggatcaagtgagagagagccggaacccagggaatgctgagttcgaagatctcacttttctagcacggtctgcactcatattgagagggtcggttgctcacaagtcctgcctgcctgcctgtgtgtatggacctgccgtagccagtgggtacgactttgaaagggagggatactctctagtcggaatagaccctttcagactgcttcaaaacagccaagtgtacagcctaatcagaccaaatgagaatccagcacacaagagtcaactggtgtggatggcatgccattctgccgcatttgaagatctaagagtattaagcttcatcaaagggacgaaggtgctcccaagagggaagctttccactagaggagttcaaattgcttccaatgaaaatatggagactatggaatcaagtacacttgaactgagaagcaggtactgggccataaggaccagaagtggaggaaacaccaatcaacagagggcatctgcgggccaaatcagcatacaacctacgttctcagtacagagaaatctcccttttgacagaacaaccgttatggcagcattcagtgggaatacagaggggagaacatctgacatgaggaccgaaatcataaggatgatggaaagtgcaagaccagaagatgtgtctttccaggggcggggagtcttcgagctctcggacgaaaaggcagcgagcccgatcgtgccttcctttgacatgagtaatgaaggatcttatttcttcggagacaatgcagaggaatacgataattaaagaaaaatacccttgtttctact